European Patent Specification EP 3 839 045 B1, published November 13, 2024. Title: Amino acid dehydrogenase mutant and use thereof. Applicant: ASYMCHEM LIFE SCIENCE(TIANJIN)CO.,LTD. Application 18930079.1. The sequence listing filed with the application follows.

SEQUENCE LISTING (2 sequences)

SEQ ID NO: 1 - protein, 301 aa, artificial sequence
  amino acid dehydrogenase
MGEKIRVAIVGYGNIGRYALDAIKAAPDMELAGVVRRSSSLGDKPAELADVPVVGSIKELTGVKVALLCTPTRSVPEYAREILALGINTVDSYDIHGQLADLRLELDKVAKEHNAVAVISAGWDPGTDSMVRCMFEFMAPKGITYTNFGPGMSMGHSVAVKAVKGVKNALSMTIPLGTGVHRRMVYVELEPGADFAQVEKAVKTDPYFVKDETHVIQVEDVDALIDMGHGVLMERKGVSGGTHNQLLSFSMRINNPALTAQIMVASARASVKQKPGAYTMIQIPIIDYMYGDPDEIIRQLV

SEQ ID NO: 2 - DNA, 906 bp, artificial sequence
  amino acid dehydrogenase gene
atgggtgaaaaaattcgcgttgcaatcgttggttacggcaacattggccgttatgccctggatgcaatcaaagccgcaccggatatggaactggccggcgtggtgcgccgtagtagcagtctgggcgacaagccggccgaactggcagatgtgcctgttgtgggcagcatcaaagagctgaccggtgtgaaagttgcactgctgtgcaccccgacccgcagtgttccggaatatgcccgtgagattctggccctgggcatcaacaccgtggatagctatgacatccacggtcagctggccgatctgcgtctggagctggataaagtggccaaagaacacaacgccgtggccgtgattagcgcaggttgggaccctggcaccgatagcatggttcgctgcatgttcgagtttatggccccgaagggcatcacctataccaatttcggtccgggcatgagcatgggtcacagcgtggccgttaaagccgtgaagggcgtgaaaaatgccctgagcatgaccattccgctgggcaccggtgttcatcgtcgtatggtgtatgtggagctggaacctggtgccgatttcgcccaggtggaaaaggccgtgaaaaccgatccgtacttcgtgaaggatgagacccacgtgattcaggtggaagacgtggacgccctgattgatatgggccatggcgttctgatggaacgtaagggcgttagcggtggcacccataaccagctgctgagcttcagtatgcgtatcaataacccggccctgaccgcccagattatggtggccagcgcccgtgccagcgtgaaacagaaaccgggcgcatacaccatgatccagattccgatcattgattacatgtacggcgacccggatgagatcattcgtcagctggtgtaa